European Patent Application EP 4 740 950 A1, published May 13, 2026. Title: Preventive or ameliorative agent for cachexia. Applicant: Osaka University. The sequence listing filed with the application follows.

SEQUENCE LISTING (8 sequences)

SEQ ID NO: 1 - DNA, 20 bp, synthetic construct
  source 1..20: mol_type = other DNA
tgatacagtcggggtgagtg

SEQ ID NO: 2 - DNA, 21 bp, synthetic construct
  source 1..21: mol_type = other DNA
aagatggtgatgggcttcccg

SEQ ID NO: 3 - DNA, 22 bp, synthetic construct
  source 1..22: mol_type = other DNA
acggaaacgacctccagacatg

SEQ ID NO: 4 - DNA, 22 bp, synthetic construct
  source 1..22: mol_type = other DNA
taccaagcctgtggtcatcctg

SEQ ID NO: 5 - DNA, 22 bp, synthetic construct
  source 1..22: mol_type = other DNA
cttctcgactgccatcctggat

SEQ ID NO: 6 - DNA, 22 bp, synthetic construct
  source 1..22: mol_type = other DNA
tcttttgggcgatgccactcag

SEQ ID NO: 7 - DNA, 21 bp, synthetic construct
  source 1..21: mol_type = other DNA
tgagtttgtccaagatggacc

SEQ ID NO: 8 - DNA, 18 bp, synthetic construct
  source 1..18: mol_type = other DNA
gccatccaggctctctgg